European Patent Application EP 4 159 760 A1, published April 5, 2023. Title: Antibody specific for CD22 and uses thereof. Applicant: InnoBation.Co., Ltd. The sequence listing filed with the application follows.

SEQUENCE LISTING (74 sequences)

SEQ ID NO: 1 - protein, 11 aa, Artificial Sequence
  1C2_VH_CDR1
GYTFTSYWMNW

SEQ ID NO: 2 - protein, 8 aa, Artificial Sequence
  1C2_VH_CDR2
IDPSDSET

SEQ ID NO: 3 - protein, 15 aa, Artificial Sequence
  1C2_VH_CDR3
ARWGNYDYDVWAMDY

SEQ ID NO: 4 - protein, 11 aa, Artificial Sequence
  1C2_VL_CDR1
QNIVHLNGNTF

SEQ ID NO: 5 - protein, 3 aa, Artificial Sequence
  1C2_VL_CDR2
KVS

SEQ ID NO: 6 - protein, 9 aa, Artificial Sequence
  1C2_VL_CDR3
FQGSHVPYT

SEQ ID NO: 7 - protein, 122 aa, Artificial Sequence
  1C2_VH_amino acid sequence
QVQLQQPGAELVRPGASVKLSCKASGYTFTSYWMNWVKQRPGQGLEWIGMIDPSDSETHYNQMFKDKATLTVDKSSSTAYMQLSSLTSEDSAVYYCARWGNYDYDVWAMDYWGQGTSVTVSS

SEQ ID NO: 8 - protein, 112 aa, Artificial Sequence
  1C2_VL_amino acid sequence
DVLMTQTPLSLPVSLGDQASISCRSSQNIVHLNGNTFLEWFLQKPGQSPKLLIYKVSNRFSGVPDRFSGSGSGTDFTLKISRVEAEDLGVYYCFQGSHVPYTFGGGTKLEIK

SEQ ID NO: 9 - DNA, 366 bp, Artificial Sequence
  1C2_VH_nucleotide sequence
caggtgcagctgcagcagcccggcgccgagctggtgaggcccggcgccagcgtgaagctgagctgcaaggccagcggctacaccttcaccagctactggatgaactgggtgaagcagaggcccggccagggcctggagtggatcggcatgatcgaccccagcgacagcgagacccactacaaccagatgttcaaggacaaggccaccctgaccgtggacaagagcagcagcaccgcctacatgcagctgagcagcctgaccagcgaggacagcgccgtgtactactgcgccaggtggggcaactacgactacgacgtgtgggccatggactactggggccagggcaccagcgtgaccgtgagcagc

SEQ ID NO: 10 - DNA, 336 bp, Artificial Sequence
  1C2_VL_nucleotide sequence
gacgtgctgatgacccagacccccctgagcctgcccgtgagcctgggcgaccaggccagcatcagctgcaggagcagccagaacatcgtgcacctgaacggcaacaccttcctggagtggttcctgcagaagcccggccagagccccaagctgctgatctacaaggtgagcaacaggttcagcggcgtgcccgacaggttcagcggcagcggcagcggcaccgacttcaccctgaagatcagcagggtggaggccgaggacctgggcgtgtactactgcttccagggcagccacgtgccctacaccttcggcggcggcaccaagctggagatcaag

SEQ ID NO: 11 - protein, 8 aa, Artificial Sequence
  9E9_VH_CDR1
GYAFSIYW

SEQ ID NO: 12 - protein, 8 aa, Artificial Sequence
  9E9_VH_CDR2
IYPGDGDT

SEQ ID NO: 13 - protein, 11 aa, Artificial Sequence
  9E9_VH_CDR3
ARRGITPWFAY

SEQ ID NO: 14 - protein, 12 aa, Artificial Sequence
  9E9_VL_CDR1
QSLLNSSNQKNY

SEQ ID NO: 15 - protein, 3 aa, Artificial Sequence
  9E9_VL_CDR2
FAS

SEQ ID NO: 16 - protein, 10 aa, Artificial Sequence
  9E9_VL_CDR3
CQQHYSTPLT

SEQ ID NO: 17 - protein, 118 aa, Artificial Sequence
  9E9_VH_amino acid sequence
EVQLEESGAELVRPGSSVKISCKASGYAFSIYWMNWVKQRPGQGLEWIGQIYPGDGDTNYNGKFKGKATLTADKSSSTAYMQLSSLTSEDSAVYFCARRGITPWFAYWGQGTLVTVSA

SEQ ID NO: 18 - protein, 113 aa, Artificial Sequence
  9E9_VL_amino acid sequence
DIVLTQSPSSLAMSVGQKVTMSCKSSQSLLNSSNQKNYLAWYQQKPGQSPKLLVYFASTRESGVPDRFIGSGSGTDFTLTISSVQAEDLADYFCQQHYSTPLTFGAGTKLELK

SEQ ID NO: 19 - DNA, 354 bp, Artificial Sequence
  9E9_VH_nucleotide sequence
gaggttcagctggaggagtctggggctgagctggtgaggcctgggtcctcagtgaagatttcctgcaaggcttctggctatgcattcagtatctactggatgaactgggtgaagcagaggcctggacagggtcttgagtggattggacagatttatcctggagatggtgatactaactacaatggaaagttcaagggtaaagccacactgactgcagacaaatcctccagcacagcctacatgcagctcagcagcctaacatctgaggactctgcggtctatttctgtgcaaggcgggggattacgccctggtttgcttactggggccaagggactctggtcactgtctctgca

SEQ ID NO: 20 - DNA, 339 bp, Artificial Sequence
  9E9_VL_nucleotide sequence
gacattgtgctgacacagtctccatcctccctggctatgtcagtaggacagaaggtcactatgagctgcaagtccagtcagagccttttaaatagtagcaatcaaaagaactatttggcctggtaccagcagaaaccaggacagtctcctaaacttctggtatactttgcatccactagggaatctggggtccctgatcgcttcataggcagtggatctgggacagatttcactcttaccatcagcagtgtgcaggctgaagacctggcagattacttctgtcagcaacattatagcactccgctcacgttcggtgctgggaccaagctggagctgaaa

SEQ ID NO: 21 - protein, 8 aa, Artificial Sequence
  2A9_VH_CDR1
GYTFTTYP

SEQ ID NO: 22 - protein, 8 aa, Artificial Sequence
  2A9_VH_CDR2
FHPYNDDT

SEQ ID NO: 23 - protein, 14 aa, Artificial Sequence
  2A9_VH_CDR3
ARGDYYVSSWYFDV

SEQ ID NO: 24 - protein, 6 aa, Artificial Sequence
  2A9_VL_CDR1
QNVGTN

SEQ ID NO: 25 - protein, 3 aa, Artificial Sequence
  2A9_VL_CDR2
SAS

SEQ ID NO: 26 - protein, 9 aa, Artificial Sequence
  2A9_VL_CDR3
QQYNSYPLT

SEQ ID NO: 27 - protein, 121 aa, Artificial Sequence
  2A9_VH_amino acid sequence
EVQLEESGAELVKPGASVKMSCKAFGYTFTTYPIEWMKQNHGKSLEWIGNFHPYNDDTKYNEKFKGKAKLTVEKSSSTVYLELSRLTSDDSAVYYCARGDYYVSSWYFDVWGAGTTVTVSS

SEQ ID NO: 28 - protein, 107 aa, Artificial Sequence
  2A9_VL_amino acid sequence
DIVMTQSQKFMSTSVGDRVSVTCKASQNVGTNVAWYQQKPGQSPKALIYSASYRYSGVPDRFTGSGSGTDFTLTISNVQSEDLAEYFCQQYNSYPLTFGSGTKLEIK

SEQ ID NO: 29 - DNA, 363 bp, Artificial Sequence
  2A9_VH_nucleotide sequence
gaggtgcagctggaggagagcggcgccgagctggtgaagcccggcgccagcgtgaagatgagctgcaaggccttcggctacaccttcaccacctaccccatcgagtggatgaagcagaaccacggcaagagcctggagtggatcggcaacttccacccctacaacgacgacaccaagtacaacgagaagttcaagggcaaggccaagctgaccgtggagaagagcagcagcaccgtgtacctggagctgagcaggctgaccagcgacgacagcgccgtgtactactgcgccaggggcgactactacgtgagcagctggtacttcgacgtgtggggcgccggcaccaccgtgaccgtgagcagc

SEQ ID NO: 30 - DNA, 321 bp, Artificial Sequence
  2A9_VL_nucleotide sequence
gacatcgtgatgacccagagccagaagttcatgagcaccagcgtgggcgacagggtgagcgtgacctgcaaggccagccagaacgtgggcaccaacgtggcctggtaccagcagaagcccggccagagccccaaggccctgatctacagcgccagctacaggtacagcggcgtgcccgacaggttcaccggcagcggcagcggcaccgacttcaccctgaccatcagcaacgtgcagagcgaggacctggccgagtacttctgccagcagtacaacagctaccccctgaccttcggcagcggcaccaagctggagatcaag

SEQ ID NO: 31 - protein, 9 aa, Artificial Sequence
  2G1_VH_CDR1
GFSLTSYDI

SEQ ID NO: 32 - protein, 7 aa, Artificial Sequence
  2G1_VH_CDR2
IWTGGGT

SEQ ID NO: 33 - protein, 12 aa, Artificial Sequence
  2G1_VH_CDR3
VPHYYGYAMDYW

SEQ ID NO: 34 - protein, 6 aa, Artificial Sequence
  2G1_VL_CDR1
QDINKY

SEQ ID NO: 35 - protein, 3 aa, Artificial Sequence
  2G1_VL_CDR2
YTS

SEQ ID NO: 36 - protein, 8 aa, Artificial Sequence
  2G1_VL_CDR3
LQYDNLLT

SEQ ID NO: 37 - protein, 117 aa, Artificial Sequence
  2G1_VH_amino acid sequence
EVQLQESGPGLVAPSQSLSITCTVSGFSLTSYDISWIRQPPGKGLEWLGVIWTGGGTNYNSAFMSRLSISKDNSKSQVFLKMNSLQTDDTAIYYCVPHYYGYAMDYWGQGTSVTVSS

SEQ ID NO: 38 - protein, 106 aa, Artificial Sequence
  2G1_VL_amino acid sequence
DIVLTQSPSSLSASLGGKVTITCKASQDINKYIAWYQHKPGKGPRLLIHYTSTLQPGIPSRFSGSGSGRDYSFSISNLEPEDIATYYCLQYDNLLTFGAGTKLELK

SEQ ID NO: 39 - DNA, 351 bp, Artificial Sequence
  2G1_VH_nucleotide sequence
gaggtgcagctgcaggagtcaggacctggcctggtggcgccctcacagagcctgtccattacctgcactgtctctgggttctcattaaccagctatgatataagctggattcgccagccaccaggaaagggtctggagtggcttggagtaatatggactggtggaggcacaaattataattcagctttcatgtccagactgagcatcagcaaggacaactccaagagccaagttttcttaaaaatgaacagtctgcaaactgatgacacagccatatattactgtgtccctcattactacggctatgctatggactactggggtcaaggaacctcagtcaccgtctcctca

SEQ ID NO: 40 - DNA, 318 bp, Artificial Sequence
  2G1_VL_nucleotide sequence
gatattgtgctgacccagtctccatcctcactgtctgcatctctgggaggcaaagtcaccatcacttgcaaggcaagccaagacattaacaagtatatagcttggtaccaacacaagcctggaaaaggtcctaggctgctcatacattacacatctacattacagccaggcatcccatcaaggttcagtggaagtgggtctgggagagattattccttcagcatcagcaacctggagcctgaagatattgcaacttattattgtctacagtatgataatctgctcacgttcggtgctgggaccaagctggagctgaaa

SEQ ID NO: 41 - protein, 8 aa, Artificial Sequence
  6B3_VH_CDR1
GYTFTDYN

SEQ ID NO: 42 - protein, 8 aa, Artificial Sequence
  6B3_VH_CDR2
IYPYNGGT

SEQ ID NO: 43 - protein, 13 aa, Artificial Sequence
  6B3_VH_CDR3
ARLYYYGRTSYWG

SEQ ID NO: 44 - protein, 6 aa, Artificial Sequence
  6B3_VL_CDR1
QNVGTY

SEQ ID NO: 45 - protein, 3 aa, Artificial Sequence
  6B3_VL_CDR2
SAS

SEQ ID NO: 46 - protein, 9 aa, Artificial Sequence
  6B3_VL_CDR3
HQYDSYPYT

SEQ ID NO: 47 - protein, 118 aa, Artificial Sequence
  6B3_VH_amino acid sequence
EVQLQQSGPELVKPGASVKISCKASGYTFTDYNMHWVKQSHGKSLEWIGYIYPYNGGTGYKQKFKSKATLTVDNSSSTAYMELRSLTSEDSAVYYCARLYYYGRTSYWGQGTTLTVSS

SEQ ID NO: 48 - protein, 107 aa, Artificial Sequence
  6B3_VL_amino acid sequence
DIVMTQSQKFMSTSVGDRVSVTCKASQNVGTYVAWYQQKPGQSPKALIYSASYRYSGVPDRFTGSGSGTDFTLTISIVQSEDLAEYFCHQYDSYPYTFGGGTKLEIK

SEQ ID NO: 49 - DNA, 354 bp, Artificial Sequence
  6B3_VH_nucleotide sequence
gaggtgcagctgcagcagagcggccccgagctggtgaagcccggcgccagcgtgaagatcagctgcaaggccagcggctacaccttcaccgactacaacatgcactgggtgaagcagagccacggcaagagcctggagtggatcggctacatctacccctacaacggcggcaccggctacaagcagaagttcaagagcaaggccaccctgaccgtggacaacagcagcagcaccgcctacatggagctgaggagcctgaccagcgaggacagcgccgtgtactactgcgccaggctgtactactacggcaggaccagctactggggccagggcaccaccctgaccgtgagcagc

SEQ ID NO: 50 - DNA, 321 bp, Artificial Sequence
  6B3_VL_nucleotide sequence
gacatcgtgatgacccagagccagaagttcatgagcaccagcgtgggcgacagggtgagcgtgacctgcaaggccagccagaacgtgggcacctacgtggcctggtaccagcagaagcccggccagagccccaaggccctgatctacagcgccagctacaggtacagcggcgtgcccgacaggttcaccggcagcggcagcggcaccgacttcaccctgaccatcagcatcgtgcagagcgaggacctggccgagtacttctgccaccagtacgacagctacccctacaccttcggcggcggcaccaagctggagatcaag

SEQ ID NO: 51 - protein, 15 aa, Artificial Sequence
  linker
GGGGSGGGGSGGGGS

SEQ ID NO: 52 - DNA, 45 bp, Artificial Sequence
  linker
ggtggtggtggttcgggtggtggtggttcgggtggtggtggttcg

SEQ ID NO: 53 - protein, 249 aa, Artificial Sequence
  1C2 scFv
DVLMTQTPLSLPVSLGDQASISCRSSQNIVHLNGNTFLEWFLQKPGQSPKLLIYKVSNRFSGVPDRFSGSGSGTDFTLKISRVEAEDLGVYYCFQGSHVPYTFGGGTKLEIKGGGGSGGGGSGGGGSQVQLQQPGAELVRPGASVKLSCKASGYTFTSYWMNWVKQRPGQGLEWIGMIDPSDSETHYNQMFKDKATLTVDKSSSTAYMQLSSLTSEDSAVYYCARWGNYDYDVWAMDYWGQGTSVTVSS

SEQ ID NO: 54 - DNA, 747 bp, Artificial Sequence
  1C2 scFv
gacgtgctgatgacccagacccccctgagcctgcccgtgagcctgggcgaccaggccagcatcagctgcaggagcagccagaacatcgtgcacctgaacggcaacaccttcctggagtggttcctgcagaagcccggccagagccccaagctgctgatctacaaggtgagcaacaggttcagcggcgtgcccgacaggttcagcggcagcggcagcggcaccgacttcaccctgaagatcagcagggtggaggccgaggacctgggcgtgtactactgcttccagggcagccacgtgccctacaccttcggcggcggcaccaagctggagatcaagggtggtggtggttcgggtggtggtggttcgggtggtggtggttcgcaggtgcagctgcagcagcccggcgccgagctggtgaggcccggcgccagcgtgaagctgagctgcaaggccagcggctacaccttcaccagctactggatgaactgggtgaagcagaggcccggccagggcctggagtggatcggcatgatcgaccccagcgacagcgagacccactacaaccagatgttcaaggacaaggccaccctgaccgtggacaagagcagcagcaccgcctacatgcagctgagcagcctgaccagcgaggacagcgccgtgtactactgcgccaggtggggcaactacgactacgacgtgtgggccatggactactggggccagggcaccagcgtgaccgtgagcagc

SEQ ID NO: 55 - protein, 246 aa, Artificial Sequence
  9E9 scFv
DIVLTQSPSSLAMSVGQKVTMSCKSSQSLLNSSNQKNYLAWYQQKPGQSPKLLVYFASTRESGVPDRFIGSGSGTDFTLTISSVQAEDLADYFCQQHYSTPLTFGAGTKLELKGGGGSGGGGSGGGGSEVQLEESGAELVRPGSSVKISCKASGYAFSIYWMNWVKQRPGQGLEWIGQIYPGDGDTNYNGKFKGKATLTADKSSSTAYMQLSSLTSEDSAVYFCARRGITPWFAYWGQGTLVTVSA

SEQ ID NO: 56 - DNA, 738 bp, Artificial Sequence
  9E9 scFv
gacattgtgctgacacagtctccatcctccctggctatgtcagtaggacagaaggtcactatgagctgcaagtccagtcagagccttttaaatagtagcaatcaaaagaactatttggcctggtaccagcagaaaccaggacagtctcctaaacttctggtatactttgcatccactagggaatctggggtccctgatcgcttcataggcagtggatctgggacagatttcactcttaccatcagcagtgtgcaggctgaagacctggcagattacttctgtcagcaacattatagcactccgctcacgttcggtgctgggaccaagctggagctgaaaggtggtggtggttcgggtggtggtggttcgggtggtggtggttcggaggttcagctggaggagtctggggctgagctggtgaggcctgggtcctcagtgaagatttcctgcaaggcttctggctatgcattcagtatctactggatgaactgggtgaagcagaggcctggacagggtcttgagtggattggacagatttatcctggagatggtgatactaactacaatggaaagttcaagggtaaagccacactgactgcagacaaatcctccagcacagcctacatgcagctcagcagcctaacatctgaggactctgcggtctatttctgtgcaaggcgggggattacgccctggtttgcttactggggccaagggactctggtcactgtctctgca

SEQ ID NO: 57 - protein, 243 aa, Artificial Sequence
  2A9 scFv
DIVMTQSQKFMSTSVGDRVSVTCKASQNVGTNVAWYQQKPGQSPKALIYSASYRYSGVPDRFTGSGSGTDFTLTISNVQSEDLAEYFCQQYNSYPLTFGSGTKLEIKGGGGSGGGGSGGGGSEVQLEESGAELVKPGASVKMSCKAFGYTFTTYPIEWMKQNHGKSLEWIGNFHPYNDDTKYNEKFKGKAKLTVEKSSSTVYLELSRLTSDDSAVYYCARGDYYVSSWYFDVWGAGTTVTVSS

SEQ ID NO: 58 - DNA, 729 bp, Artificial Sequence
  2A9 scFv
gacatcgtgatgacccagagccagaagttcatgagcaccagcgtgggcgacagggtgagcgtgacctgcaaggccagccagaacgtgggcaccaacgtggcctggtaccagcagaagcccggccagagccccaaggccctgatctacagcgccagctacaggtacagcggcgtgcccgacaggttcaccggcagcggcagcggcaccgacttcaccctgaccatcagcaacgtgcagagcgaggacctggccgagtacttctgccagcagtacaacagctaccccctgaccttcggcagcggcaccaagctggagatcaagggtggtggtggttcgggtggtggtggttcgggtggtggtggttcggaggtgcagctggaggagagcggcgccgagctggtgaagcccggcgccagcgtgaagatgagctgcaaggccttcggctacaccttcaccacctaccccatcgagtggatgaagcagaaccacggcaagagcctggagtggatcggcaacttccacccctacaacgacgacaccaagtacaacgagaagttcaagggcaaggccaagctgaccgtggagaagagcagcagcaccgtgtacctggagctgagcaggctgaccagcgacgacagcgccgtgtactactgcgccaggggcgactactacgtgagcagctggtacttcgacgtgtggggcgccggcaccaccgtgaccgtgagcagc

SEQ ID NO: 59 - protein, 238 aa, Artificial Sequence
  2G1 scFv
DIVLTQSPSSLSASLGGKVTITCKASQDINKYIAWYQHKPGKGPRLLIHYTSTLQPGIPSRFSGSGSGRDYSFSISNLEPEDIATYYCLQYDNLLTFGAGTKLELKGGGGSGGGGSGGGGSEVQLQESGPGLVAPSQSLSITCTVSGFSLTSYDISWIRQPPGKGLEWLGVIWTGGGTNYNSAFMSRLSISKDNSKSQVFLKMNSLQTDDTAIYYCVPHYYGYAMDYWGQGTSVTVSS

SEQ ID NO: 60 - DNA, 714 bp, Artificial Sequence
  2G1 scFv
gatattgtgctgacccagtctccatcctcactgtctgcatctctgggaggcaaagtcaccatcacttgcaaggcaagccaagacattaacaagtatatagcttggtaccaacacaagcctggaaaaggtcctaggctgctcatacattacacatctacattacagccaggcatcccatcaaggttcagtggaagtgggtctgggagagattattccttcagcatcagcaacctggagcctgaagatattgcaacttattattgtctacagtatgataatctgctcacgttcggtgctgggaccaagctggagctgaaaggtggtggtggttcgggtggtggtggttcgggtggtggtggttcggaggtgcagctgcaggagtcaggacctggcctggtggcgccctcacagagcctgtccattacctgcactgtctctgggttctcattaaccagctatgatataagctggattcgccagccaccaggaaagggtctggagtggcttggagtaatatggactggtggaggcacaaattataattcagctttcatgtccagactgagcatcagcaaggacaactccaagagccaagttttcttaaaaatgaacagtctgcaaactgatgacacagccatatattactgtgtccctcattactacggctatgctatggactactggggtcaaggaacctcagtcaccgtctcctca

SEQ ID NO: 61 - protein, 239 aa, Artificial Sequence
  6B3 scFv
DIVMTQSQKFMSTSVGDRVSVTCKASQNVGTYVAWYQQKPGQSPKALIYSASYRYSGVPDRFTGSGSGTDFTLTISIVQSEDLAEYFCHQYDSYPYTFGGGTKLEIGGGGSGGGGSGGGGSEVQLQQSGPELVKPGASVKISCKASGYTFTDYNMHWVKQSHGKSLEWIGYIYPYNGGTGYKQKFKSKATLTVDNSSSTAYMELRSLTSEDSAVYYCARLYYYGRTSYWGQGTTLTVSS

SEQ ID NO: 62 - DNA, 720 bp, Artificial Sequence
  6B3 scFv
gacatcgtgatgacccagagccagaagttcatgagcaccagcgtgggcgacagggtgagcgtgacctgcaaggccagccagaacgtgggcacctacgtggcctggtaccagcagaagcccggccagagccccaaggccctgatctacagcgccagctacaggtacagcggcgtgcccgacaggttcaccggcagcggcagcggcaccgacttcaccctgaccatcagcatcgtgcagagcgaggacctggccgagtacttctgccaccagtacgacagctacccctacaccttcggcggcggcaccaagctggagatcaagggtggtggtggttcgggtggtggtggttcgggtggtggtggttcggaggtgcagctgcagcagagcggccccgagctggtgaagcccggcgccagcgtgaagatcagctgcaaggccagcggctacaccttcaccgactacaacatgcactgggtgaagcagagccacggcaagagcctggagtggatcggctacatctacccctacaacggcggcaccggctacaagcagaagttcaagagcaaggccaccctgaccgtggacaacagcagcagcaccgcctacatggagctgaggagcctgaccagcgaggacagcgccgtgtactactgcgccaggctgtactactacggcaggaccagctactggggccagggcaccaccctgaccgtgagcagc

SEQ ID NO: 63 - DNA, 1178 bp, Artificial Sequence
  EF1 promoter
gctccggtgcccgtcagtgggcagagcgcacatcgcccacagtccccgagaagttggggggaggggtcggcaattgaaccggtgcctagagaaggtggcgcggggtaaactgggaaagtgatgtcgtgtactggctccgcctttttcccgagggtgggggagaaccgtatataagtgcagtagtcgccgtgaacgttctttttcgcaacgggtttgccgccagaacacaggtaagtgccgtgtgtggttcccgcgggcctggcctctttacgggttatggcccttgcgtgccttgaattacttccacctggctgcagtacgtgattcttgatcccgagcttcgggttggaagtgggtgggagagttcgaggccttgcgcttaaggagccccttcgcctcgtgcttgagttgaggcctggcctgggcgctggggccgccgcgtgcgaatctggtggcaccttcgcgcctgtctcgctgctttcgataagtctctagccatttaaaatttttgatgacctgctgcgacgctttttttctggcaagatagtcttgtaaatgcgggccaagatctgcacactggtatttcggtttttggggccgcgggcggcgacggggcccgtgcgtcccagcgcacatgttcggcgaggcggggcctgcgagcgcggccaccgagaatcggacgggggtagtctcaagctggccggcctgctctggtgcctggcctcgcgccgccgtgtatcgccccgccctgggcggcaaggctggcccggtcggcaccagttgcgtgagcggaaagatggccgcttcccggccctgctgcagggagctcaaaatggaggacgcggcgctcgggagagcgggcgggtgagtcacccacacaaaggaaaagggcctttccgtcctcagccgtcgcttcatgtgactccactgagtaccgggcgccgtccaggcacctcgattagttctcgagcttttggagtacgtcgtctttaggttggggggaggggttttatgcgatggagtttccccacactgagtgggtggagactgaagttaggccagcttggcacttgatgtaattctccttggaatttgccctttttgagtttggatcttggttcattctcaagcctcagacagtggttcaaagtttttttcttccatttcaggtgtcgtga

SEQ ID NO: 64 - DNA, 63 bp, Artificial Sequence
  signal peptide
atggccttaccagtgaccgccttgctcctgccgctggccttgctgctccacgccgccaggccg

SEQ ID NO: 65 - DNA, 135 bp, Artificial Sequence
  CD8 Hinge
accacgacgccagcgccgcgaccaccaacaccggcgcccaccatcgcgtcgcagcccctgtccctgcgcccagaggcgtgccggccagcggcggggggcgcagtgcacacgagggggctggacttcgcctgtgat

SEQ ID NO: 66 - DNA, 72 bp, Artificial Sequence
  TM
atctacatctgggcgcccttggccgggacttgtggggtccttctcctgtcactggttatcaccctttactgc

SEQ ID NO: 67 - DNA, 126 bp, Artificial Sequence
  4-1BB
aaacggggcagaaagaaactcctgtatatattcaaacaaccatttatgagaccagtacaaactactcaagaggaagatggctgtagctgccgatttccagaagaagaagaaggaggatgtgaactg

SEQ ID NO: 68 - DNA, 336 bp, Artificial Sequence
  CD3zeta
agagtgaagttcagcaggagcgcagacgcccccgcgtacaagcagggccagaaccagctctataacgagctcaatctaggacgaagagaggagtacgatgttttggacaagagacgtggccgggaccctgagatggggggaaagccgagaaggaagaaccctcaggaaggcctgtacaatgaactgcagaaagataagatggcggaggcctacagtgagattgggatgaaaggcgagcgccggaggggcaaggggcacgatggcctttaccagggtctcagtacagccaccaaggacacctacgacgcccttcacatgcaggccctgccccctcgc

SEQ ID NO: 69 - DNA, 591 bp, Artificial Sequence
  WPRE
atcaacctctggattacaaaatttgtgaaagattgactggtattcttaactatgttgctccttttacgctatgtggatacgctgctttaatgcctttgtatcatgctattgcttcccgtatggctttcattttctcctccttgtataaatcctggttgctgtctctttatgaggagttgtggcccgttgtcaggcaacgtggcgtggtgtgcactgtgtttgctgacgcaacccccactggttggggcattgccaccacctgtcagctcctttccgggactttcgctttccccctccctattgccacggcggaactcatcgccgcctgccttgcccgctgctggacaggggctcggctgttgggcactgacaattccgtggtgttgtcggggaagctgacgtcctttccatggctgctcgcctgtgttgccacctggattctgcgcgggacgtccttctgctacgtcccttcggccctcaatccagcggaccttccttcccgcggcctgctgccggctctgcggcctcttccgcgtcttcgccttcgccctcagacgagtcggatctccctttgggccgcctccccgcctg

SEQ ID NO: 70 - protein, 21 aa, Artificial Sequence
  signal peptide
MALPVTALLLPLALLLHAARP

SEQ ID NO: 71 - protein, 45 aa, Artificial Sequence
  CD8 Hinge
TTTPAPRPPTPAPTIASQPLSLRPEACRPAAGGAVHTRGLDFACD

SEQ ID NO: 72 - protein, 24 aa, Artificial Sequence
  TM
IYIWAPLAGTCGVLLLSLVITLYC

SEQ ID NO: 73 - protein, 42 aa, Artificial Sequence
  4-1BB
KRGRKKLLYIFKQPFMRPVQTTQEEDGCSCRFPEEEEGGCEL

SEQ ID NO: 74 - protein, 112 aa, Artificial Sequence
  CD3zeta
RVKFSRSADAPAYKQGQNQLYNELNLGRREEYDVLDKRRGRDPEMGGKPRRKNPQEGLYNELQKDKMAEAYSEIGMKGERRRGKGHDGLYQGLSTATKDTYDALHMQALPPR